European Patent Application EP 4 293 041 A1, published December 20, 2023. Title: AMPLIFICATION ENHANCER AND USE THEREOF. Applicant: CURE GENETICS CO., LIMITED. The sequence listing filed with the application follows.

SEQUENCE LISTING (15 sequences)

SEQ ID NO: 1 - protein, 486 aa, Artificial Sequence
  CJP molecule
MALPVTALLLPLALLLHAARPDIQMTQTTSSLSASLGDRVTISCRASQDISKYLNWYQQKPDGTVKLLIYHTSRLHSGVPSRFSGSGSGTDYSLTISNLEQEDIATYFCQQGNTLPYTFGGGTKLEITGGGGSGGGGSGGGGSEVKLQESGPGLVAPSQSLSVTCTVSGVSLPDYGVSWIRQPPRKGLEWLGVIWGSETTYYNSALKSRLTIIKDNSKSQVFLKMNSLQTDDTAIYYCAKHYYYGGSYAMDYWGQGTSVTVSSTTTPAPRPPTPAPTIASQPLSLRPEACRPAAGGAVHTRGLDFACDIYIWAPLAGTCGVLLLSLVITLYCKRGRKKLLYIFKQPFMRPVQTTQEEDGCSCRFPEEEEGGCELRVKFSRSADAPAYKQGQNQLYNELNLGRREEYDVLDKRRGRDPEMGGKPRRKNPQEGLYNELQKDKMAEAYSEIGMKGERRRGKGHDGLYQGLSTATKDTYDALHMQALPPR

SEQ ID NO: 2 - protein, 482 aa, Artificial Sequence
  C7R sequence
SLDNNGTATPELPTQGTFSNVSTNVSYQETTTPSTLGSTSLHPVSQHGNEATTNITETTVKFTSTSVITSVYGNTNSSVQSQTSVISTVFTTPANVSTPETTLKPSLSPGNVSDLSTTSTSLATSPTKPYTSSSPILSDIKAEIKCSGIREVKLTQGICLEQNKTSSCAEFKKDRGEGLARVLCGEEQADADAGAQVCSLLLAQSEVRPQCLLLVLANRTEISSKLQLMKKHQSDLKKLGILDFTEQDVASHQSYSQKTPILLTCPTISILSFFSVALLVILACVLWKKRIKPIVWPSLPDHKKTLEHLCKKPRKNLNVSFNPESFLDCQIHRVDDIQARDEVEGFLQDTFPQQLEESEKQRLGGDVQSPNCPSEDVVITPESFGRDSSLTCLAGNVSACDAPILSSSRSLDCRESGKNGPHVYQDLLLSLGTTNSTLPPPFSLQSGILTLNPVAQGQPILTSLGSNQEEAYVTMSSFYQNQ

SEQ ID NO: 3 - protein, 241 aa, Artificial sequence
  Enhancer
LRPVQAQAQSDCSCSTVSPILLTCPTISILSFFSVALLVILACVLWKKRIKPIVWPSLPDHKKTLEHLCKKPRKNLNVSFNPESFLDCQIHRVDDIQARDEVEGFLQDTFPQQLEESEKQRLGGDVQSPNCPSEDVVITPESFGRDSSLTCLAGNVSACDAPILSSSRSLDCRESGKNGPHVYQDLLLSLGTTNSTLPPPFSLQSGILTLNPVAQGQPILTSLGSNQEEAYVTMSSFYQNQ

SEQ ID NO: 4 - protein, 245 aa, Artificial Sequence
  Enhancer
LRPVQAQAQSDCSCSTVSPILLTCPTISILSFFSVALLVILACVLWKKRIKPIVWPSLPDHKKTLEHLCKKPRKNLNVSFNPESFLDCQIHRVDDIQARDEVEGFLQDTFPQQLEESEKQRLGGDVQSPNCPSEDVVITPESFGRDSSLTCLAGNVSACDAPILSSSRSLDCRESGKNGPHVYQDLLLSLGTTNSTLPPPFSLQSGILTLNPVAQGQPILTSLGSNQEEAYVTMSSFYRHQVPSV

SEQ ID NO: 5 - protein, 251 aa, Artificial Sequence
  Enhancer
LRPVQAQAQSDCSCSTVSPILLTCPTISILSFFSVALLVILACVLWKKRIKPIVWPSLPDHKKTLEHLCKKPRKNLNVSFNPESFLDCQIHRVDDIQARDEVEGFLQDTFPQQLEESEKQRLGGDVQSPNCPSEDVVITPESFGRDSSLTCLAGNVSACDAPILSSSRSLDCRESGKNGPHVYQDLLLSLGTTNSTLPPPFSLQSGILTLNPVAQGQPILTSLGSNQEEAYVTMSSFYQNQSGYRHQVPSV

SEQ ID NO: 6 - protein, 266 aa, Artificial Sequence
  Enhancer
LRPVQAQAQSDCSCSTVSPILLTCPTISILSFFSVALLVILACVLWKKRIKPIVWPSLPDHKKTLEHLCKKPRKNLNVSFNPESFLDCQIHRVDDIQARDEVEGFLQDTFPQQLEESEKQRLGGDVQSPNCPSEDVVITPESFGRDSSLTCLAGNVSACDAPILSSSRSLDCRESGKNGPHVYQDLLLSLGTTNSTLPPPFSLQSGILTLNPVAQGQPILTSLGSNQEEAYVTMSSFYQNQSQNTSSTVQYSTVVHSGYRHQVPSV

SEQ ID NO: 7 - protein, 143 aa, Artificial Sequence
  chimeric molecule
MSRSVALAVLALLSLSGLEAVMAPRTVLLGGGGSGGGGSGGGGSIQRTPKIQVYSRHPAENGKSNFLNCYVSGFHPSDIEVDLLKNGERIEKVEHSDLSFSKDWSFYLLYYTEFTPTEKDEYACRVNHVTLSQPKIVKWDRDM

SEQ ID NO: 8 - RNA, 109 nt, Artificial Sequence
  sgRNA
cucacgcuggauagccuccguuuuagagcuaugcuggaaacagcauagcaaguuaaaauaaggcuaguccguuaucaacuugaaaaaguggcaccgagucggugcuuuu

SEQ ID NO: 9 - RNA, 109 nt, Artificial Sequence
  sgRNA
aguagcgcgagcacagcuaguuuuagagcuaugcuggaaacagcauagcaaguuaaaauaaggcuaguccguuaucaacuugaaaaaguggcaccgagucggugcuuuu

SEQ ID NO: 10 - RNA, 99 nt, Artificial Sequence
  sgRNA
gagucucucagcugguacaguuuuagagcuagaaauagcaaguuaaaauaaggcuaguccguuaucaacuugaaaaaguggcaccgagucggugcuuuu

SEQ ID NO: 11 - protein, 25 aa, Artificial Sequence
  transmembrane domain
PILLTISILSFFSVALLVILACVLW

SEQ ID NO: 12 - protein, 19 aa, Artificial Sequence
  P2A linker
ATNFSLLKQAGDVEENPGP

SEQ ID NO: 13 - protein, 18 aa, Artificial Sequence
  T2A linker
EGRGSLLTCGDVEENPGP

SEQ ID NO: 14 - protein, 21 aa, Artificial Sequence
  Signal
MGGLEPCSRLLLLPLLLAVSG

SEQ ID NO: 15 - protein, 242 aa, Artificial Sequence
  Enhancer
LRPVQAQAQSDCSCSTVSPGVLAGIVMGDLVLTVLIALAVYFLKKRIKPIVWPSLPDHKKTLEHLCKKPRKNLNVSFNPESFLDCQIHRVDDIQARDEVEGFLQDTFPQQLEESEKQRLGGDVQSPNCPSEDVVITPESFGRDSSLTCLAGNVSACDAPILSSSRSLDCRESGKNGPHVYQDLLLSLGTTNSTLPPPFSLQSGILTLNPVAQGQPILTSLGSNQEEAYVTMSSFYRHQVPSV